European Patent Specification EP 3 518 669 B1, published March 1, 2023. Title: ANIMAL MODEL OF ANGELMAN SYNDROME. Applicant: University of South Florida The Regents of the University of California The Texas A&M University System Weeber, Edwin John Segal, David J. O'Geen, Henriette Pyles, Benjamin Dindot, Scott V. The sequence listing filed with the application follows.

SEQUENCE LISTING (26 sequences)

SEQ ID NO: 1 - protein, 875 aa, Homo sapiens
MEKLHQCYWKSGEPQSDDIEASRMKRAAAKHLIERYYHQLTEGCGNEACTNEFCASCPTFLRMDNNAAAIKALELYKINAKLCDPHPSKKGASSAYLENSKGAPNNSCSEIKMNKKGARIDFKDVTYLTEEKVYEILELCREREDYSPLIRVIGRVFSSAEALVQSFRKVKQHTKEELKSLQAKDEDKDEDEKEKAACSAAAMEEDSEASSSRIGDSSQGDNNLQKLGPDDVSVDIDAIRRVYTRLLSNEKIETAFLNALVYLSPNVECDLTYHNVYSRDPNYLNLFIIVMENRNLHSPEYLEMALPLFCKAMSKLPLAAQGKLIRLWSKYNADQIRRMMETFQQLITYKVISNEFNSRNLVNDDDAIVAASKCLKMVYYANVVGGEVDTNHNEEDDEEPIPESSELTLQELLGEERRNKKGPRVDPLETELGVKTLDCRKPLIPFEEFINEPLNEVLEMDKDYTFFKVETENKFSFMTCPFILNAVTKNLGLYYDNRIRMYSERRITVLYSLVQGQQLNPYLRLKVRRDHIIDDALVRLEMIAMENPADLKKQLYVEFEGEQGVDEGGVSKEFFQLVVEEIFNPDIGMFTYDESTKLFWFNPSSFETEGQFTLIGIVLGLAIYNNCILDVHFPMVVYRKLMGKKGTFRDLGDSHPVLYQSLKDLLEYEGNVEDDMMITFQISQTDLFGNPMMYDLKENGDKIPITNENRKEFVNLYSDYILNKSVEKQFKAFRRGFHMVTNESPLKYLFRPEEIELLICGSRNLDFQALEETTEYDGGYTRDSVLIREFWEIVHSFTDEQKRLFLQFTTGTDRAPVGGLGKLKMIIAKNGPDTERLPTSHTCFNVLLLPEYSSKEKLKERLLKAITYAKGFGML

SEQ ID NO: 2 - DNA, 4491 bp, Homo sapiens
acagatcaggagaacctcagtctgacgacattgaagctagccgaatgaagcgagcagctgcaaagcatctaatagaacgctactaccaccagttaactgagggctgtggaaatgaagcctgcacgaatgagttttgtgcttcctgtccaacttttcttcgtatggataataatgcagcagctattaaagccctcgagctttataagattaatgcaaaactctgtgatcctcatccctccaagaaaggagcaagctcagcttaccttgagaactcgaaaggtgcccccaacaactcctgctctgagataaaaatgaacaagaaaggcgctagaattgattttaaagatgtgacttacttaacagaagagaaggtatatgaaattcttgaattatgtagagaaagagaggattattcccctttaatccgtgttattggaagagttttttctagtgctgaggcattggtacagagcttccggaaagttaaacaacacaccaaggaagaactgaaatctcttcaagcaaaagatgaagacaaagatgaagatgaaaaggaaaaagctgcatgttctgctgctgctatggaagaagactcagaagcatcttcctcaaggataggtgatagctcacagggagacaacaatttgcaaaaattaggccctgatgatgtgtctgtggatattgatgccattagaagggtctacaccagattgctctctaatgaaaaaattgaaactgcctttctcaatgcacttgtatatttgtcacctaacgtggaatgtgacttgacgtatcacaatgtatactctcgagatcctaattatctgaatttgttcattatcgtaatggagaatagaaatctccacagtcctgaatatctggaaatggctttgccattattttgcaaagcgatgagcaagctaccccttgcagcccaaggaaaactgatcagactgtggtctaaatacaatgcagaccagattcggagaatgatggagacatttcagcaacttattacttataaagtcataagcaatgaatttaacagtcgaaatctagtgaatgatgatgatgccattgttgctgcttcgaagtgcttgaaaatggtttactatgcaaatgtagtgggaggggaagtggacacaaatcacaatgaagaagatgatgaagagcccatccctgagtccagcgagctgacacttcaggaacttttgggagaagaaagaagaaacaagaaaggtcctcgagtggaccccctggaaactgaacttggtgttaaaaccctggattgtcgaaaaccacttatcccttttgaagagtttattaatgaaccactgaatgaggttctagaaatggataaagattatacttttttcaaagtagaaacagagaacaaattctcttttatgacatgtccctttatattgaatgctgtcacaaagaatttgggattatattatgacaatagaattcgcatgtacagtgaacgaagaatcactgttctctacagcttagttcaaggacagcagttgaatccatatttgagactcaaagttagacgtgaccatatcatagatgatgcacttgtccggctagagatgatcgctatggaaaatcctgcagacttgaagaagcagttgtatgtggaatttgaaggagaacaaggagttgatgagggaggtgtttccaaagaattttttcagctggttgtggaggaaatcttcaatccagatattggtatgttcacatacgatgaatctacaaaattgttttggtttaatccatcttcttttgaaactgagggtcagtttactctgattggcatagtactgggtctggctatttacaataactgtatactggatgtacattttcccatggttgtctacaggaagctaatggggaaaaaaggaacttttcgtgacttgggagactctcacccagttctatatcagagtttaaaagatttattggagtatgaagggaatgtggaagatgacatgatgatcactttccagatatcacagacagatctttttggtaacccaatgatgtatgatctaaaggaaaatggtgataaaattccaattacaaatgaaaacaggaaggaatttgtcaatctttattctgactacattctcaataaatcagtagaaaaacagttcaaggcttttcggagaggttttcatatggtgaccaatgaatctcccttaaagtacttattcagaccagaagaaattgaattgcttatatgtggaagccggaatctagatttccaagcactagaagaaactacagaatatgacggtggctataccagggactctgttctgattagggagttctgggaaatcgttcattcatttacagatgaacagaaaagactcttcttgcagtttacaacgggcacagacagagcacctgtgggaggactaggaaaattaaagatgattatagccaaaaatggcccagacacagaaaggttacctacatctcatacttgctttaatgtgcttttacttccggaatactcaagcaaagaaaaacttaaagagagattgttgaaggccatcacgtatgccaaaggatttggcatgctgtaaaacaaaacaaaacaaaataaaacaaaaaaaaggaaggaaaaaaaaagaaaaaatttaaaaaattttaaaaatataacgagggataaatttttggtggtgatagtgtcccagtacaaaaaggctgtaagatagtcaaccacagtagtcacctatgtctgtgcctcccttctttattggggacatgtgggctggaacagcagatttcagctacatatatgaacaaatcctttattattattataattatttttttgcgtgaaagtgttacatattctttcacttgtatgtacagagaggtttttctgaatatttattttaagggttaaatcacttttgcttgtgtttattactgcttgaggttgagccttttgagtatttaaaaaatatataccaacagaactactctcccaaggaaaatattgccaccatttgtagaccacgtaaccttcaagtatgtgctacttttttgtccctgtatctaactcaaatcaggaactgtattttttttaatgatttgcttttgaaacttgaagtcttgaaaacagtgtgatgcaattactgctgttctagcccccaaagagttttctgtgcaaaatcttgagaatcaatcaataaagaaagatggaaggaagggagaaattggaatgttttaactgcagccctcagaactttagtaacagcacaacaaattaaaaacaaaaacaactcatgccacagtatgtcgtcttcatgtgtcttgcaatgaactgtttcagtagccaatcctctttcttagtatatgaaaggacagggatttttgttcttgttgttctcgttgttgttttaagtttactggggaaagtgcatttggccaaatgaaatggtagtcaagcctattgcaacaaagttaggaagtttgttgtttgtttattataaacaaaaagcatgtgaaagtgcacttaagatagagtttttattaattacttacttattacctagattttaaatagacaatccaaagtctccccttcgtgttgccatcatcttgttgaatcagccattttatcgaggcacgtgatcagtgttgcaacataatgaaaaagatggctactgtgccttgtgttacttaatcatacagtaagctgacctggaaatgaatgaaactattactcctaagaattacattgtatagccccacagattaaatttaattaattaattcaaaacatgttaaacgttactttcatgtactatggaaaagtacaagtaggtttacattactgatttccagaagtaagtagtttcccctttcctagtcttctgtgtatgtgatgttgttaatttcttttattgcattataaaataaaaggattatgtatttttaactaaggtgagacattgatatatccttttgctacaagctatagctaatgtgctgagcttgtgccttggtgattgattgattgattgactgattgttttaactgattactgtagatcaacctgatgatttgtttgtttgaaattggcaggaaaaatgcagctttcaaatcattggggggagaaaaaggatgtctttcaggattattttaattaatttttttcataattgagacagaactgtttgttatgtaccataatgctaaataaaactgtggcacttttcaccataatttaatttagtggaaaaagaagacaatgctttccatattgtgataaggtaacatggggtttttctgggccagcctttagaacactgttagggtacatacgctaccttgatgaaagggaccttcgtgcaactgtagtcatcttaaaggcttctcatccactgtgcttcttaatgtgtaattaaagtgaggagaaattaaatactctgagggcgttttatataataaattcgtgaaga

SEQ ID NO: 3 - protein, 868 aa, Rattus norvegicus
MATACKRSSGESQSEDIEASRMKRAAAKHLIERYYHQLTEGCGNEACTNEFCASCPTFLRMDNNAAAIKALELYKINAKLCDPHPSKKGASSAYLENSKGASNNSEIKMNKKEEFKEVDYLTEEKVYEIYEFCREREDYSPLIRVIGRIFSSAEALVQSFRKVKQHTKEELKSLQEKDEDKDEDEKEKAACSAAAMEEDSEASSSRMGDSSQGDNNVQKLGPDDVTVDIDAIRRVYSSLLSDEKIETAFLNALVYLSPNVECDLTYHNVYTRDPNYLNLFIIVMENRNLHSPEYLEMALPLFCKAMSKLPLAAQGKLIRLWSKYSADQIRRMMETFQQLITYKVISNEFNSRNLVNDDDAIVAASKCLKMVYYANVVGGDVDTNHNEEDDEEPIPESSELTLQELLGEERRNKKGPRVDPLETEIGVKTLDCRKPLISFEEFINEPLNDVLEMDKDYTFFKVETENKFSFMTCPFILNAVTKNLGLYYDNRIRMYSERRITVLYSLVQGQQLNPYLRLKVRRDHIIDDALVRLEMIAMENPADLKKQLYVEFEGEQGVDEGGVSKEFFQLVVEEIFNPDIGMFTYDEATRLFWFNPSSFETEGQFTLIGIVLGLAIYNNCILDVHFPMVVYRKLMGKKGTFCDLGDSHPILYQSLKDLLEYEGNVEDDMMITFQISQTDLFGNPMMYDLKENGDKIPITNENRKEFVSLYSDYILNKSVEKQFKAFRRGFHMVTNESPLKYLFRPEEIELLICGSRNLDFQALEETTEYDGGYTRESVVIREFWEIVHSFTDEQKRLFLQFTTGTDRAPVGGLGKLKMIIAKNGPDTERLPTSHTCFNVLLLPEYSSKEKLKERLLKAITYAKGFGML

SEQ ID NO: 4 - DNA, 5795 bp, Rattus norvegicus
gtcgggatactcggtccgcccacctagtcttctcgtcctcgttcgcgagatccgtgtttctcccaagatggtggcgctcctctttgggtgactacaggagacgacagggcctttcgtcttcgcaagtacctcgccgcccctcctgcgttcgctcgcgcaccgggccacgcagctgttcaccgcctcatcacgactctcctcgttcgaccagtcgcggacggtggcgcctccttctgcttctcttcggagttgctcgccaccctcgccccccaccgtggacagatcgcggcagcagccgttcagcgccgacttcaaggttgcccaggcgcccggcctcccggcctcagtttcctgaggagaagcgcgggtcccgcatgagacccggcggtggcgccagcgaaagggaacgaggcggtggcgggcggcggcggtggacgagggcgacaaggaccagtgaggcggccgcagctgcgagggccgcagcccacgcgcgggggcgaggacaggttaaaaatctgtaagagcctgattttagagttcaccagctcctcagaagtttggcgaaatatgaattattaagcctacgttcagatcaagttagcagctagactggtgtgacaacctgtttttaatcagtgactcaaagctgttatcaccctgatgtcaccgaatggccacagcttgtaaaagatcatcaggagaatcccagtctgaggacattgaagctagccgaatgaagcgagcagctgcaaagcatctaatagagcgctactaccatcagttaactgagggctgtggaaatgaggcctgcacgaatgagttctgtgcttcctgtccaacttttcttcgtatggataacaatgcagcagctattaaagctcttgagctttataaaattaatgcaaaactctgtgatcctcatccctccaagaaaggagcaagctcagcttaccttgagaactcaaaaggtgcatctaacaactcagagataaaaatgaacaagaaggaagagtttaaagaggtggactacctaactgaagagaaagtatatgaaatttatgaattttgtagggagagagaggattactcccctttaattcgtgtaattggaagaatattttctagtgctgaggcactggttcagagctttcggaaagtcaaacagcacactaaggaggaattgaaatctcttcaagagaaggatgaagacaaggatgaagatgaaaaggaaaaagctgcgtgttctgctgctgctatggaagaagactcagaagcatcttcttcaaggatgggtgatagctcacagggagacaacaatgtacaaaaattaggtcctgatgatgtgactgtggatattgatgctataagaagggtctacagcagtttgctctctgatgaaaaaatagaaactgccttcctgaatgcacttgtatatctgtcacctaacgtggaatgtgatttgacatatcataatgtgtacactcgagaccctaattatctcaatttgttcattattgtaatggaaaataggaatctccacagtcctgaatatctggaaatggcattgccgttattttgcaaagctatgagtaagctaccccttgcagctcaaggaaaactgattaggctgtggtctaaatacagtgctgaccagattcggagaatgatggaaacatttcagcaacttattacctacaaagtcataagcaatgaatttaatagccgaaatctagtgaatgatgatgatgccattgttgctgcttcaaagtgtttgaaaatggtttactatgcaaatgtagtgggaggggacgtggacacaaatcataatgaggaagatgatgaagagcctatacctgagtccagtgaattgacacttcaggagcttctgggagaggaaagaagaaataagaaaggtcctcgagtggatccactagaaaccgaaattggcgttaaaactctagattgtcgaaaaccacttatctcctttgaagaattcattaatgaaccactgaatgatgttctagaaatggacaaagattatacttttttcaaagttgaaacagagaacaaattctcttttatgacatgtccctttatattgaatgctgtcacaaagaatctgggattgtattatgacaatagaattcgcatgtacagtgaaagaagaatcactgttctttacagcctagttcaaggacagcagttgaatccatatttgagacttaaagtcagacgtgaccatattatagatgatgcacttgtccggctagagatgatcgctatggaaaatcctgcagacttgaagaaacagttgtatgtggaatttgaaggagaacaaggagtagatgagggaggcgtttccaaagagttttttcagttggttgtggaggaaatctttaatccagatattggtatgttcacatacgatgaagctacaagattattttggtttaatccatcttcttttgaaactgagggtcaatttactctgattggcatagtcctgggtctggctatttacaataactgtatactggatgtccattttcccatggttgtgtacaggaagctaatggggaaaaaaggaacgttttgtgacttgggagactctcacccaatcttatatcagagtttaaaggatttattggaatatgaagggaatgtggaagatgatatgatgatcactttccagatatcacagacagatctttttggtaacccaatgatgtatgatctaaaagaaaatggtgataaaattccaattacaaatgaaaacaggaaggaatttgtcagtctctattcagactacattctcaataaatctgtagaaaaacaattcaaggcatttcgcagaggttttcatatggtgactaatgaatcacccttaaaatacttattcagaccagaagaaattgaattacttatatgtggaagccggaatctcgatttccaggcactagaagaaactacagagtatgatggtggctatacgagagaatctgttgtgattagggagttctgggaaattgttcattcgtttacagatgaacagaaaagacttttcctgcagtttacaacaggcacagacagagcacctgttggaggactcggaaaattgaagatgattatagccaaaaatggcccagacacagaaaggttacctacatctcatacttgctttaatgtccttttacttccggaatattcaagcaaagaaaaacttaaagagagattgctgaaggccatcacatatgccaaaggatttggcatgctgtaaacaaaacaaaaacaaaaagaaaaaaagaaaaaagtcaaaaaacttaataaatataagagggataatttgatggtaatagtgtcccagttcaaaaaggctgtaagatagtgaaccacagtactcatctatgtctgtgcctcccttcttcattggggacattgtgggctggaacagcagatttcagctgcatatatgaacaaatcctttattattattataattatttttttgcgtgaaagtgttacatattctttcacttgtatgtacagagaggtttttctgaatatttattttaagggttaaatcacttttgcttgtgtttattactgcttgaggttgagcctttttgagtatttaaaatatatataccaacgaaactattctcgcaaggaaaacattgccaccatttgtagaccatgtaatcttcaagtatgtgtttttttttggccctgtatctaagtcaaatcaggaacttttttttaaccatttgcttttgaaacttgaagttaaggaaacagtgtggtgcaagtactgctgttctagcccccaaggagttttctgtacaaaattttgagaatcaataaagatggaagggagaatttggaatgtttgaaccacagccctcagaactttagtaacagcacaacaaattaaaacaactcatgccacagtacgttgtcttcatgtgtcttgcaatgaactgtttcagtagccaatccttttagtatatgaaaggacagggatcttttttattgttgttgttgttgttgttgttgttgttgttgtttttgttgtttaagtttactggggaaagtgcatctggccaaatgataggatagtcaagcctattgcaacaaaattagaaagtttgttgtataaataagcatgtaaaagtgcacttaaaatgaatctttattattcccgagattttaaatagacaatccaaagtctccccttctcttgccatcatcttgtttaatcaactatttttcaaggcactcgatcagtgttgcagcataatagaaagtccagctactgtgccttgtgttatttatttacacagtaaacaggcctggaaatgaatggaactagtactcctgagaattaaattgtatatcctccaaattaaaatttacttcaaaagtgttaaagaattcatgtcctatatataaaatacaaataggcttagattgctggacatttaatgtagtttcccatccctagtcttttatgtttgtgatgttaatttcttttgttgcataacaaaataaaagaattatgtatttttaactaaggagagacatactggtatatcattttactacaagctacagatatcctgttgagcttgtgccttgattgttttcacaactagtacaaatcaacctgatgttttaaattggcagggaataattaattgtagctttcaaatcattggaaggggaaaaggatgtcttttaggattattttccttcttgtagtagttgaggcagagctattatttactgtaatgctaaatgaaacagtggcttaaatactttaatgggaaaaaagaacacagtgcgttccatattgtgataaggtaatgtgaggtttttccttttttttctgagctagcctttagaacactgttgtggtatgtatgctaccttgattataggaccccctaaatgtgactatagtcatcataatgggcatctagtccactgtgcttcttatgtattatgaaagtgataagaagacaaattaagtgggtatattttataaaataaattcatgaagagatttgtgttcttcagttctcaagtttattatcactacagtattgaagtagttgtgatactatatctgtgtgaaagttttgaaatggtaatatagattatcaaacagaagtaacatcagtatatttaaaagaaagtgaaaacaaataaacctaaaatgttttcagaggtaaaaatacattctcacttgcttcctagtcagtttttcttggcatgttgccacattattatggctgccttttcatcattgcttttctagattgtcatggaacaatatttccgagttaaaaaaatacctcttgctatagtagaacatttcaaaattacagcataaaagcacagtctggagcaaaatttttctggagacttggcagctgcagcaaacaaattgagtgtctgtacatattgtggtctataagttaattgtgtgatcaaattcatttgtaataaccttacctttatttggaagtacatccctgtgtaggaacgtatatatcaaaagaaacctataaatgagggttcagagaaccggttcatattgacatgtggcacatgcatcactgggcagcatcactccctgtttccataaggtggctatgctgaaatcaacctcttaaagaattattttctcaagaatccatataacctagaaaaagaagtgttttactgaggctactctttctgatgttcatcctttaacttcttatcccaagacttatttttatcctttctaccct

SEQ ID NO: 5 - protein, 872 aa, Macaca mulatta
MATACKRSGEPQSDDIEASRMKRAAAKHLIERYYHQLTEGCGNEACTNEFCASCPTFLRMDNNAAAIKALELYKINAKLCDPHPSKKGASSAYLENSKGAPNNSCSEIKMNKKGTRIDFKDVTYLTEEKVYEILELCREREDYSPLIRVIGRVFSSAEALVQSFRKVKQHTKEELKSLQAKDEDKDEDEKEKAACSAAAMEEDSEASSSRIGDSSQGDNNLQKVGPDDVSVDIDAIRRVYTRLLSNEKIETAFLNALVYLSPNVECDLTYHNVYSRDPNYLNLFIIVMENRNLHSPEYLEMALPLFCKAMSKLPLAAQGKLIRLWSKYNADQIRRMMETFQQLITYKVISNEFNSRNLVNDDDAIVAASKCLKMVYYANVVGGEVDTNHNEEDDEEPIPESSELTLQELLGEERRNKKGPRVDPLETELGVKTLDCRKPLIPFEEFINEPLNEVLEMDKDYTFFKVETENKFSFMTCPFILNAVTKNLGLYYDNRIRMYSERRITVLYSLVQGQQLNPYLRLKVRRDHIIDDALVRLEMIAMENPADLKKQLYVEFEGEQGVDEGGVSKEFFQLVVEEIFNPDIGMFTYDESTKLFWFNPSSFETEGQFTLIGIVLGLAIYNNCILDVHFPMVVYRKLMGKKGTFRDLGDSHPVLYQSLKDLLEYEGNVEDDMMITFQISQTDLFGNPMMYDLKENGDKIPITNENRKEFVNLYSDYILNKSVEKQFKAFRRGFHMVTNESPLKYLFRPEEIELLICGSRNLDFQALEETTEYDGGYTRDSVLIREFWEIVHSFTDEQKRLFLQFTTGTDRAPVGGLGKLKMIIAKNGPDTERLPTSHTCFNVLLLPEYSSKEKLKERLLKAITYAKGFGML

SEQ ID NO: 6 - DNA, 2882 bp, Macaca mulatta
gcggaggcggcgggcgagggcgacgacgaccagtgaggcggccgccgcagcccaggcgcgggggcgacgacaggttaaaaatctgtaagagcctgattttagaattcaccagctcctcagaagtttggcgaaatatgagttattaagcctacgctcagatcaaggtagcagctagactggtgtgacaacctgtttttaatcagtgactcaaagctgtgatcaccctgatgtcaccgaatggccacagcttgtaaaagatcaggagaacctcagtctgacgacattgaagctagccgaatgaagcgagcagctgcaaagcatctaatagaacgctactaccaccagttaactgagggctgtggaaatgaagcctgcacgaatgagttttgtgcttcctgtccaacttttcttcgtatggataataatgcagcagctattaaagccctcgagctttataagattaatgcaaaactctgtgatcctcatccctccaagaaaggagcaagctcagcttaccttgagaactcgaaaggtgcccccaacaactcctgctctgagataaaaatgaacaagaaaggcactagaattgattttaaagatgtgacttacttaacagaagagaaggtatatgaaattcttgaattatgtagagaaagagaggattattcccctttaattcgtgttattggaagagttttttctagtgctgaggcattggtacagagcttccggaaagttaaacaacataccaaggaagaactgaaatctcttcaagcaaaagatgaagacaaggatgaagatgaaaaggaaaaagctgcatgttctgctgctgctatggaagaagactcagaagcatcttcctcaaggataggtgatagctcacagggagacaacaatttgcagaaagtaggccctgatgatgtgtctgtggatattgatgccattagaagggtctacaccagattgctgtctaatgaaaaaattgaaactgcctttctcaatgcacttgtatatttgtcacctaacgtggaatgtgacttgacgtatcacaatgtatactctcgagatcctaattatctgaatttgttcattatcgtaatggagaatagaaatctccacagtcctgaatatctggaaatggctttgccattattttgcaaagcaatgagcaagctaccccttgcagcccaaggaaaactgatcagactgtggtctaaatacaatgcagaccagattcggagaatgatggagacatttcagcaacttattacttacaaagtcataagcaatgaatttaacagtcgaaatctagtgaacgatgatgatgccattgttgctgcttcgaagtgcttgaaaatggtttactatgcaaatgtagtgggaggggaagtggacacaaatcacaatgaagaagatgatgaagagcccatccctgaatccagtgagctgacacttcaggagcttttgggagaagaaagaagaaacaagaaaggtcctcgagtggaccccctggaaactgaacttggtgttaaaaccctggattgtcgaaaaccacttatcccttttgaagagtttattaatgaaccactgaatgaggttctagaaatggataaagattatacttttttcaaagtagaaacagagaacaaattctcttttatgacatgtccctttatattaaatgctgtcacaaagaatttgggattatattatgacaatagaattcgcatgtacagtgaacgaagaatcactgttctctacagcttagttcaaggacagcagttgaatccatatttgagactcaaagttagacgtgaccatatcatagatgatgcacttgtccggctagagatgatcgctatggaaaatcctgcagacttgaagaagcagttgtatgtggaatttgaaggagaacaaggagttgatgaaggaggtgtttccaaagaattttttcagctggttgtggaggaaatcttcaatccagatattggtatgttcacatacgatgaatctacaaaattgttttggtttaatccgtcttcttttgaaactgagggtcagtttactctgattggcatagtactgggtctggctatttacaataactgtatactggatgtacattttcccatggttgtctacagaaagctaatggggaaaaaaggaacttttcgtgacttgggagactctcacccagttctgtatcagagtttaaaagatttattggagtatgaagggaatgtggaagacgacatgatgatcactttccagatatcacagacagatctttttggtaacccaatgatgtatgatctaaaggaaaatggtgataaaattccaattacaaatgaaaacaggaaggaatttgtcaatctttattctgactacattctcaataaatcagtagaaaaacagttcaaggcttttcggagaggttttcatatggtgaccaatgaatctcccttaaagtacttattcagaccagaagaaattgaattgcttatatgtggaagccggaatctagatttccaagcattagaagaaactacagaatatgacggtggctataccagggactctgttctgattagggagttctgggaaatcgttcattcatttacagatgaacagaaaagactcttcttgcagtttacaacgggcacagacagagcacctgtgggaggactaggaaaattaaagatgattatagccaaaaatggcccagacacagaaaggttacctacatctcatacttgctttaatgtgcttttacttccggaatattcaagcaaagaaaaacttaaagagagattgttgaaggccatcacgtatgccaaaggatttggcatgctgtaaaacaaaacaaaataaaacaaaaaaaa

SEQ ID NO: 7 - protein, 856 aa, Xenopus tropicalis
MKRAAAKHLIERYYHQLTEGCGNETCTNEFCASCPTFLRMDNNAAAIKALELYKVNAKLCDPHPSKKGTSSSYLENNSKSAHNNSCTERKMNKKDLHGPRDDFKDVTFLSEEKVYEILELCREKEDYSPLIRVIGRVFSSAEALVQSFRKAKHHTKEELKSLQEKDEDKDEDEKEKAASSAAAMEEDSGASSSRLSDNSQGDNNIQKLGPEEVSLDIEAVRRVYHRLLSNEKIETAFLNALVYLSPNVECDLTYHNVYSRDPNYLNLFIIVMENGNLHSPEYLEMALPLFCKAMSKLPLAAQAKLIRLWSKYSAEQIRRMMETFQQLITYKVISNEFNSRNLVNDDDAIVAATKCLKMVYYSNVVGGEIETDHNEEEDDEPVPESSELTLQELLGEERRNKKGPRVDPLETELGVKSIDCRKPLIPFEEFVNEPLNDVLEMDKDYTFFKVETENKFSFMTCPFILNAVTKNLGLYYDNRIRMYSERRITVLYSLVQGQQLNPYLRLKVRRDHIIDDALVRLEMIAMENPADLKKQLYVEFEGEQGVDEGGVSKEFFQLVVEEIFNPDIGMFTYDESTKHSWFNPSSFETEGQFTLIGIVLGLAIYNNCILDVHFPMVVYRKLMGKKGTFRDLADSHPVLYQSLKELLEYEGNVEEDMMMTFQISQTDLFGNPLMHDLKENGDKIPITNENRKEFVSLYTDYILNKSVEKQFKAFRRGFHMVTNESPLKYLFRPEEIELLICGSRNLDFQALKDTTEYDGGYTRDSNIIKEFWEIVNSFTEEQKRLFLQFTTGTDRAPVGGLGKLKMIIAKNGPDTDRLPTSHTCFNVLLLPEYSNKEKLKERLLKAITYAKGFGML

SEQ ID NO: 8 - DNA, 2948 bp, Xenopus tropicalis
ctctcgcgagatgagacttttgacgtcgggattagctgtccggcaggggccaggaatctgggtattatcggcgttgcgggacgtttaagcagcaatctgggactgcgggctgtgtttaaaaattcgggtgtgttgggcggtatgcagtagtgctgtggtttagattgggggtctcgcatgagttccccggacaagaggtggcagcaggagagagagggagccccggagcccgaggagaggaggaccaacaccccccgcagcagcccgggacacagccctgaaggagacagatcaccaggagacccttattcagaaaatctagaaaatagccgaatgaagcgagcagctgcaaagcatctaatagaacgctactaccaccagttaactgagggttgtggaaatgaaacctgcacgaatgaattttgtgcttcctgtcccacttttcttcgtatggataacaatgcagcagccattaaggccctcgagttatataaggttaatgcaaaactctgtgatcctcatccctccaagaaaggaacaagctcatcttatctagagaacaattcgaaaagtgcccataacaactcctgcacagaaagaaagatgaataagaaagaccttcatggacccagagatgactttaaagatgtcactttcctgtctgaagaaaaagtgtatgaaattcttgaattgtgtagagaaaaagaggactactcgcctttaattcgggtgatcgggagagtattttccagtgcagaagctttggttcagagtttccgaaaagcaaagcaccatacaaaggaggagctaaaatccttgcaagaaaaggatgaagataaggatgaagatgaaaaggaaaaagctgcatcatctgctgctgcaatggaagaggattctggagcatcatcctcaaggttaagtgacaactcacaaggagacaacaacatacagaaactaggccctgaagaagtgtctctagatatagaagcagttcgacgggtgtatcacaggttactttctaatgagaaaatagaaactgcctttctgaatgcacttgtgtacctttctcctaatgtggaatgtgacttaacttatcataatgtttattcacgagatcccaactatctcaatttgtttataatcgtcatggagaatggtaatctccatagtcctgaatacctggaaatggctttaccgttgttttgcaaagcaatgagtaaattgccattagcagcgcaagcaaagttgatccgtctttggtcaaagtacagcgctgagcagattcgccgaatgatggaaacatttcagcagcttataacctataaagttataagtaacgagttcaacagtcgaaatttagtcaatgatgatgatgctattgttgcagcaacaaagtgcttaaaaatggtttactattcaaatgttgttggtggagagattgaaactgaccataatgaagaggaagatgatgaacctgttcctgagtccagtgagttaactctgcaggagctgctaggggaagaacgaagaaacaaaaaaggccctcgagtagatccccttgaaaccgaacttggtgttaaaagcattgattgcaggaaacctctcatccctttcgaggaattcgttaacgaaccactaaatgatgttctagaaatggacaaagattatactttctttaaagtagagactgaaaacaaattctcttttatgacttgcccctttatcctgaatgcagttacaaagaatcttggtctgtattatgacaacagaatccgcatgtacagtgaaaggcgaataactgttctgtatagtctagtgcaaggacagcaacttaacccctatttgaggctcaaagtacggcgagatcacatcattgacgatgctcttgttaggcttgagatgattgccatggaaaatcctgcagatttgaagaagcaattatatgtggaatttgagggagaacaaggagttgacgaaggaggtgtttctaaagagtttttccaattagttgttgaagaaattttcaaccctgatattggtatgtttacgtatgatgagtccactaaacactcttggttcaatccatcatcttttgagacagaaggacagtttacacttattggcattgtgctgggccttgcaatttacaataattgcattctagatgtgcattttccaatggttgtatatagaaaactaatggggaaaaaaggaaccttccgtgaccttgctgattctcatcctgttctttatcagagtttaaaagaattgttggagtatgaaggcaatgttgaagaagatatgatgatgactttccagatctctcagactgacctctttggaaatcctttaatgcacgacttaaaggaaaatggagataaaatccccattacaaatgagaacagaaaggaatttgtcagtctatacacagactatattctaaataaatcagtggaaaagcaatttaaagccttcagaaggggctttcacatggttaccaatgaatcgcctctgaaatatctgtttagaccagaggagattgaacttcttatttgtggaagtaggaatttagatttccaagctctgaaagatactacggaatatgatggtggctataccagagattcaaatataataaaggagttttgggaaattgtaaattctttcacagaggaacaaaaaagattgttcttgcaatttacaacaggcacggacagagcacctgtaggtgggctaggcaaattaaagatgattatagccaaaaacggccctgatacagacaggttaccaacatctcatacttgctttaatgtccttttgcttccggagtactcaaataaagagaaactgaaggagagattgttaaaggccatcacttatgctaaggggtttggtatgctctaaaaacaaaggcaagcgtgctaaaaaaaaataaaaaaaaaaaaaaa

SEQ ID NO: 9 - protein, 857 aa, Danio rerio
MKRAAAKHLIERYYHQLTEGCGNEACTNEACGSSPGFQRMDNNAAAIKALELYKNNAKLCDPHPSKKGASSAFPENSAKGAHNFSACSNGKMNHKDLPPTREDFRDLNFLTEDKVYEILSICSETEDYSPLIRVIGRVFSSAESLVQSFRKAKQHTKEELKSLQAKDEDKDEDEKETASGSSTAMEVEPEASASSGDGSSHGENNVQKLGPVEVSVDIDAVRRVYDRLLSNEKIEAAFLNALVYLSPNVECDLTYHNVYAADPNYLNVFIIVMENSNLHSPEYLEIALPQFCKAMSKLPLPALAKLARLWSQYGVDQIRRLVETFQQLITYTVISNEFSSDNLVNEDDGVVAATKCLKIVYYANVLGGDLDTDHNEEDDDEPIPESSELTLQELLGEERRNKKGPRVDPLETEMGIRASDCRKPLIPFEEFINEPLNEVLEMDKDYTFFKVETESKFSFMTCPFILNAVTKNLGLYYDNRIRMYSERRITALYSLVQGQQLNPYLRLKVRRDHIIDDALVRLEMIAMENPADLKKQLYVEFEGEQGVDEGGVSKEFFQLVVEEIFNPDIGMFTYDESTKLFWFNPSSFENEGQFTLIGIVLGLAIYNNCILDVHFPMVIYRKLMGKKGTFRDLADSHPVLFQSLKDLMEYEGNVEEDMMITFQISQTDLFGNPLMYDLKESGDKIPVTNENRKDFVALYAEYMLNKSVEKQFKAFRRGFHMVTNESPLKYLFRPEEIELLICGSRNLDFQALEESTEYDGGYNKDSRIIRDFWETVHSFEQEKKRLFLQFTTGTDRAPVGGLGKLKMIIAKNGPDSDRLPTSHTCFNVLLLPEYSTVEKLKERLLKAITYAKGFGML

SEQ ID NO: 10 - DNA, 4093 bp, Danio rerio
caagatggccgcgaatattttgtggaggggttggagttgaatacacgccgcactagaagcgattgtgatgttgagagaccagattcattcgtcagcatcagaacacctccaaaagattgctacctgacaacctttgggtctctttgagttcagaaccgtagaagagtgtgatattggaaactttaaagcaagtctaatgaagcgagcggctgcaaagcatttaattgagcgctactaccaccagttaacagagggctgtggaaatgaggcctgcacgaatgaggcttgtggctcttctccgggtttccagcgcatggataacaatgcagcagccatcaaggccctggagttatataagaataatgccaaactgtgtgatcctcatccctctaagaaaggagccagttcagccttcccggagaacagtgccaaaggagctcacaacttctctgcttgcagcaacggaaagatgaaccataaggacctgccacccacaagggaggactttagagatctgaatttcttgactgaggataaggtgtatgaaatcctgagcatctgcagtgagacagaggactattctcctctaatccgtgttattggtcgggttttctcaagtgcagagagtctagtccagagtttccgcaaagcaaaacaacacaccaaggaagagctcaagtcccttcaggccaaggatgaagacaaagatgaagatgagaaagaaacggcttctggttcatccacagcaatggaggtggaaccagaagcttcagcatcaagtggagacgggtcatctcatggggagaacaacgtccaaaagttgggtcctgtagaagtttctgtagacattgatgctgtaagaagagtgtacgacagattattatcgaatgagaagattgaggcagctttcctcaacgcgttagtctatttgtcgcccaacgtagagtgtgacctcacctatcacaatgtgtacgccgctgaccctaattacctgaacgtcttcatcattgtgatggagaacagtaacctccacagtcccgaatacttagaaatcgccttgccacagttctgcaaggccatgagcaagctacctcttccggctctggccaagcttgcacggttgtggtcgcagtacggtgtggaccagatccgacgtttggtcgagactttccagcagcttattacctacacggtcatcagcaacgagttcagcagtgataacctagtcaatgaggatgatggtgtggtggcagccaccaagtgcttgaaaatcgtctactatgcaaacgtgctgggcggcgacctagacacggatcacaatgaggaggacgacgatgaaccgatccctgagtcaagtgagctgacgctgcaggagctgctgggagaggagagacgcaataaaaaaggccctcgagtggatccgctggagacagaaatgggcatccgtgcctcggactgtcgaaaacccctcatcccattcgaggagttcatcaatgaaccactcaatgaggtgctggaaatggacaaagactataccttcttcaaggtggagacagagagcaagttctcctttatgacctgccctttcatacttaacgctgtgactaagaatctgggcctgtactacgacaaccggatccgcatgtatagcgagcgcaggattactgccctctatagtttggtgcaaggacagcaactaaacccttatctgcgactcaaagtgcgcagagaccacatcatagacgatgctcttgtcaggttggagatgattgccatggaaaaccctgcagacttgaagaagcaactgtatgtggagtttgagggtgagcaaggagtagatgagggaggagtatccaaagaattctttcaactggtagtagaggagatcttcaacccagatataggcatgtttacctatgatgaaagcacaaaacttttctggttcaacccttcatcatttgagaatgaaggccagttcactttgataggcatcgtcctgggcctagctatctacaataactgcattctggatgtgcatttccctatggtgatttacagaaaactaatgggaaagaaaggaacgtttcgagaccttgcagactctcatccggttctttttcagagtctgaaagatctcatggagtatgaaggcaatgttgaagaagacatgatgattaccttccagatctcgcaaacagacctgtttggaaacccactaatgtacgatttaaaggaaagcggtgataaaatccctgttaccaatgagaacagaaaggattttgtggcgctctatgcagagtacatgctgaacaaaagtgtggagaaacagtttaaggcctttagaagaggattccacatggtcactaatgagtctccactgaaatatctgtttcgaccggaggagattgagctgcttatatgtggcagcaggaaccttgacttccaagcacttgaagagagcaccgaatatgatggaggatacaacaaagactcgcgcattattagggatttctgggagacggtgcactcatttgagcaggagaagaagagactgtttctccagttcaccactggcacagatagagctccagttggaggtttaggcaaactcaagatgattattgccaaaaatggtcccgactcagacaggttacccacctctcatacctgcttcaacgtgctgctcctccccgaatactccaccgtggagaaacttaaagagagactccttaaagccatcacttacgccaaaggcttcggcatgctctgaggctaaagaactcactctagccctcagaggagaatcagctacatccacaactaatcgtaaatatcaagtttaaatgtaaggcaacatgaaatgggttcaaaatggggaagttctggtgaccgtgtgcctgtgcctaaaaagtagataaaaccacactggactcatggctctctctctttctctgtctctctctctctccctcttatgtaagtgttcaggttcccatttttttgtatgcactgagatatagcgttatttattttaagggatgaaatctcttgtcatgtctgccaggaattccacacttttgttgcttcatagtcataaaaacaggagggacggttggaagttttcaacggctgcaggactgatcaccaactaaacttaataaaacaagatcaaagggaggaggtggaactttgttgtattacggttgaactgtgaaagtgcacttaactctattcagaatgtctttgttttatttttgatttttttttgtcaacccttaggcttttctttttagttttggctcgtgcttcattggtcttccctagttcgttcacatttgcggcaatgtttgaaaggtacagagcagcctcagtctcagtttggcatccaggaatctgtatttattgagaatctgcattgtttgtaatgccgtcgtgctgctcgtttatggccagtgttctgcatttcgcttcagattcgactttttctctccctcacacacaactgaccggtttgctaaagatcacagtggtgcactcctgccgaaaacgagtagtgttataaaggagagatctcaacttcctataaaactctgtcagaagcttcctactagtgtttgtttgttttgttatctgtcttgttttaattcaagatggcagacttttagtccatgaatgctaattgacggtgccccatgaagaaagcgttttagttgcgcttttttttttctttgctctgcacagtgtctggcccgatacatttggatgaaaatgaggggaaattggcacaagtcgtaccactatcttgtcgtgccaaacagttatgctgagaatcgccgctccggttttgttcaggcgtagctggaaatccagattagtgatgccctgttcactttttttttttttgtttattttgtttttccttattccctcttgcagattaaatgtgactgtggtttgatccactgctgatggcgctaacataaaagggggaaacagaacttgatattgagaatgacaacatttgattgtttcaagttattcttaaataaattcaaaactgaaaaacaaaaaaaaaaaaaaaaaaaaaaaaaaa

SEQ ID NO: 11 - DNA, 20 bp, Rattus norvegicus
ggccctgcagagatgcaatc

SEQ ID NO: 12 - DNA, 17 bp, Rattus norvegicus
ggagccctccgccggca

SEQ ID NO: 13 - DNA, 17 bp, Rattus norvegicus
tacccttcccaggcccc

SEQ ID NO: 14 - DNA, 20 bp, Rattus norvegicus
gcatttctagtacatcatcc

SEQ ID NO: 15 - DNA, 20 bp, Artificial
  Ub3aDelF1 forward primer
aacaccaagcctctctcagc

SEQ ID NO: 16 - DNA, 20 bp, Artificial
  Ub3aDelR1 reverse primer
accaggcctcaaaattgaca

SEQ ID NO: 17 - DNA, 20 bp, Artificial
  Ub3aDelF2 forward primer
ctcccgagtacaccgaagac

SEQ ID NO: 18 - DNA, 20 bp, Artificial
  Ub3aDelR2 reverse primer
gggaacagcaaaagacatgg

SEQ ID NO: 19 - DNA, 22 bp, Artificial
  Ub3aDelSpcfcF3 forward primer
gtaccaagaagtcacatggctc

SEQ ID NO: 20 - DNA, 23 bp, Artificial
  Ub3aDelSpcfcR3 reverse primer
gcaggctgctattacactaagga

SEQ ID NO: 21 - DNA, 23 bp, Artificial
  Ub3aDelSpcfcF4 forward primer
acatggctctaaaagagttcagg

SEQ ID NO: 22 - DNA, 23 bp, Artificial
  Ub3aDelSpcfcR4 reverse primer
gtgattcactagggatatgcagg

SEQ ID NO: 23 - RNA, 24 nt, Rattus norvegicus
uugugauucugaacaguucuuggg

SEQ ID NO: 24 - RNA, 22 nt, Rattus norvegicus
agcacuguacuacuaggggcuc

SEQ ID NO: 25 - DNA, 67 bp, Rattus norvegicus
ccaagagcgaaggcgaactagagtagggccctgcagagattaaataaatcccaggccccccagaatt

SEQ ID NO: 26 - DNA, 67 bp, Rattus norvegicus
ccaagagcgaaggcgaactagagtagggccccgcagaattaaataattgatgatgatgatgatgatg